European Patent Application EP 4 799 643 A1, published September 2, 2026. Title: 一种药物组合物及其用途. Applicant: 苏州瑞博生物技术股份有限公司. Application WO. The sequence listing filed with the application follows.

SEQUENCE LISTING (26 sequences)

SEQ ID NO: 1 - RNA, 19 nt, synthetic construct
  source 1..19: mol_type = other RNA
  misc_feature 19: note = n is a; note (original language) = n为a
  misc_feature 1..19: note = synthetic sequence; note (original language) = 合成序列
ccttgaggcatacttcaan

SEQ ID NO: 2 - RNA, 19 nt, synthetic construct
  source 1..19: mol_type = other RNA
  misc_feature 1: note = n is u; note (original language) = n为u
  misc_feature 1..19: note = synthetic sequence; note (original language) = 合成序列
nttgaagtatgcctcaagg

SEQ ID NO: 3 - RNA, 19 nt, synthetic construct
  source 1..19: mol_type = other RNA
  misc_feature 19: note = n is a; note (original language) = n为a
  misc_feature 1..19: note = synthetic sequence; note (original language) = 合成序列
gtgtgcacttcgcttcacn

SEQ ID NO: 4 - RNA, 19 nt, synthetic construct
  source 1..19: mol_type = other RNA
  misc_feature 1: note = n is u; note (original language) = n为u
  misc_feature 1..19: note = synthetic sequence; note (original language) = 合成序列
ngtgaagcgaagtgcacac

SEQ ID NO: 5 - RNA, 19 nt, synthetic construct
  source 1..19: mol_type = other RNA
  misc_feature 19: note = n is u; note (original language) = n为u
  misc_feature 1..19: note = synthetic sequence; note (original language) = 合成序列
ggacttctctcaattttcn

SEQ ID NO: 6 - RNA, 19 nt, synthetic construct
  source 1..19: mol_type = other RNA
  misc_feature 1: note = n is a; note (original language) = n为a
  misc_feature 1..19: note = synthetic sequence; note (original language) = 合成序列
ngaaaattgagagaagtcc

SEQ ID NO: 7 - RNA, 19 nt, synthetic construct
  source 1..19: mol_type = other RNA
  misc_feature 19: note = n is a; note (original language) = n为a
  misc_feature 1..19: note = synthetic sequence; note (original language) = 合成序列
ctgtaggcataaattggtn

SEQ ID NO: 8 - RNA, 19 nt, synthetic construct
  source 1..19: mol_type = other RNA
  misc_feature 1: note = n is u; note (original language) = n为u
  misc_feature 1..19: note = synthetic sequence; note (original language) = 合成序列
naccaatttatgcctacag

SEQ ID NO: 9 - RNA, 17 nt, synthetic construct
  source 1..17: mol_type = other RNA
  misc_feature 17: note = n is a; note (original language) = n为a
  misc_feature 1..17: note = synthetic sequence; note (original language) = 合成序列
gtgcacttcgcttcacn

SEQ ID NO: 10 - RNA, 19 nt, synthetic construct
  source 1..19: mol_type = other RNA
  misc_feature 1: note = n is u; note (original language) = n为u
  misc_feature 1..19: note = synthetic sequence; note (original language) = 合成序列
naccaatttatgcctacag

SEQ ID NO: 11 - RNA, 19 nt, synthetic construct
  source 1..19: mol_type = other RNA
  modified_base 1: mod_base = OTHER; note = Methoxy modification; note (original language) = 甲氧基修饰
  modified_base 1..2: mod_base = OTHER; note = Thiophosphate ester subunit connection; note (original language) = 硫代磷酸酯亚基连接
  modified_base 2: mod_base = OTHER; note = Methoxy modification; note (original language) = 甲氧基修饰
  modified_base 2..3: mod_base = OTHER; note = Thiophosphate ester subunit connection; note (original language) = 硫代磷酸酯亚基连接
  modified_base 3: mod_base = OTHER; note = Methoxy modification; note (original language) = 甲氧基修饰
  modified_base 4: mod_base = OTHER; note = Methoxy modification; note (original language) = 甲氧基修饰
  modified_base 5: mod_base = OTHER; note = Methoxy modification; note (original language) = 甲氧基修饰
  modified_base 6: mod_base = OTHER; note = Methoxy modification; note (original language) = 甲氧基修饰
  modified_base 7: mod_base = OTHER; note = Fluorinated modification; note (original language) = 氟代修饰
  modified_base 8: mod_base = OTHER; note = Fluorinated modification; note (original language) = 氟代修饰
  modified_base 9: mod_base = OTHER; note = Fluorinated modification; note (original language) = 氟代修饰
  modified_base 10: mod_base = OTHER; note = Methoxy modification; note (original language) = 甲氧基修饰
  modified_base 11: mod_base = OTHER; note = Methoxy modification; note (original language) = 甲氧基修饰
  modified_base 12: mod_base = OTHER; note = Methoxy modification; note (original language) = 甲氧基修饰
  modified_base 13: mod_base = OTHER; note = Methoxy modification; note (original language) = 甲氧基修饰
  modified_base 14: mod_base = OTHER; note = Methoxy modification; note (original language) = 甲氧基修饰
  modified_base 15: mod_base = OTHER; note = Methoxy modification; note (original language) = 甲氧基修饰
  modified_base 16: mod_base = OTHER; note = Methoxy modification; note (original language) = 甲氧基修饰
  modified_base 17: mod_base = OTHER; note = Methoxy modification; note (original language) = 甲氧基修饰
  modified_base 18: mod_base = OTHER; note = Methoxy modification; note (original language) = 甲氧基修饰
  modified_base 19: mod_base = OTHER; note = Methoxy modification; note (original language) = 甲氧基修饰
  misc_feature 1..19: note = synthetic sequence; note (original language) = 合成序列
ccttgaggcatacttcaaa

SEQ ID NO: 12 - RNA, 21 nt, synthetic construct
  source 1..21: mol_type = other RNA
  modified_base 1: mod_base = OTHER; note = 5'-(E)-vinylphosphonate (E-VP) modification; note (original language) = 乙烯基磷酸酯修饰
  modified_base 1: mod_base = OTHER; note = Methoxy modification; note (original language) = 甲氧基修饰
  modified_base 1..2: mod_base = OTHER; note = Thiophosphate ester subunit connection; note (original language) = 硫代磷酸酯亚基连接
  modified_base 2: mod_base = OTHER; note = Fluorinated modification; note (original language) = 氟代修饰
  modified_base 2..3: mod_base = OTHER; note = Thiophosphate ester subunit connection; note (original language) = 硫代磷酸酯亚基连接
  modified_base 3: mod_base = OTHER; note = Methoxy modification; note (original language) = 甲氧基修饰
  modified_base 4: mod_base = OTHER; note = Methoxy modification; note (original language) = 甲氧基修饰
  modified_base 5: mod_base = OTHER; note = Methoxy modification; note (original language) = 甲氧基修饰
  modified_base 6: mod_base = OTHER; note = Fluorinated modification; note (original language) = 氟代修饰
  modified_base 7: mod_base = OTHER; note = Methoxy modification; note (original language) = 甲氧基修饰
  modified_base 8: mod_base = OTHER; note = Methoxy modification; note (original language) = 甲氧基修饰
  modified_base 9: mod_base = OTHER; note = Methoxy modification; note (original language) = 甲氧基修饰
  modified_base 10: mod_base = OTHER; note = Methoxy modification; note (original language) = 甲氧基修饰
  modified_base 11: mod_base = OTHER; note = Methoxy modification; note (original language) = 甲氧基修饰
  modified_base 12: mod_base = OTHER; note = Methoxy modification; note (original language) = 甲氧基修饰
  modified_base 13: mod_base = OTHER; note = Methoxy modification; note (original language) = 甲氧基修饰
  modified_base 14: mod_base = OTHER; note = Fluorinated modification; note (original language) = 氟代修饰
  modified_base 15: mod_base = OTHER; note = Methoxy modification; note (original language) = 甲氧基修饰
  modified_base 16: mod_base = OTHER; note = Fluorinated modification; note (original language) = 氟代修饰
  modified_base 17: mod_base = OTHER; note = Methoxy modification; note (original language) = 甲氧基修饰
  modified_base 18: mod_base = OTHER; note = Methoxy modification; note (original language) = 甲氧基修饰
  modified_base 19: mod_base = OTHER; note = Methoxy modification; note (original language) = 甲氧基修饰
  modified_base 19..20: mod_base = OTHER; note = Thiophosphate ester subunit connection; note (original language) = 硫代磷酸酯亚基连接
  modified_base 20: mod_base = OTHER; note = Methoxy modification; note (original language) = 甲氧基修饰
  modified_base 20..21: mod_base = OTHER; note = Thiophosphate ester subunit connection; note (original language) = 硫代磷酸酯亚基连接
  modified_base 21: mod_base = OTHER; note = Methoxy modification; note (original language) = 甲氧基修饰
  misc_feature 1..21: note = synthetic sequence; note (original language) = 合成序列
tttgaagtatgcctcaaggtt

SEQ ID NO: 13 - RNA, 19 nt, synthetic construct
  source 1..19: mol_type = other RNA
  modified_base 1: mod_base = OTHER; note = Methoxy modification; note (original language) = 甲氧基修饰
  modified_base 1..2: mod_base = OTHER; note = Thiophosphate ester subunit connection; note (original language) = 硫代磷酸酯亚基连接
  modified_base 2: mod_base = OTHER; note = Methoxy modification; note (original language) = 甲氧基修饰
  modified_base 2..3: mod_base = OTHER; note = Thiophosphate ester subunit connection; note (original language) = 硫代磷酸酯亚基连接
  modified_base 3: mod_base = OTHER; note = Methoxy modification; note (original language) = 甲氧基修饰
  modified_base 4: mod_base = OTHER; note = Methoxy modification; note (original language) = 甲氧基修饰
  modified_base 5: mod_base = OTHER; note = Fluorinated modification; note (original language) = 氟代修饰
  modified_base 6: mod_base = OTHER; note = Methoxy modification; note (original language) = 甲氧基修饰
  modified_base 7: mod_base = OTHER; note = Fluorinated modification; note (original language) = 氟代修饰
  modified_base 8: mod_base = OTHER; note = Fluorinated modification; note (original language) = 氟代修饰
  modified_base 9: mod_base = OTHER; note = Fluorinated modification; note (original language) = 氟代修饰
  modified_base 10: mod_base = OTHER; note = Methoxy modification; note (original language) = 甲氧基修饰
  modified_base 11: mod_base = OTHER; note = Methoxy modification; note (original language) = 甲氧基修饰
  modified_base 12: mod_base = OTHER; note = Methoxy modification; note (original language) = 甲氧基修饰
  modified_base 13: mod_base = OTHER; note = Methoxy modification; note (original language) = 甲氧基修饰
  modified_base 14: mod_base = OTHER; note = Methoxy modification; note (original language) = 甲氧基修饰
  modified_base 15: mod_base = OTHER; note = Methoxy modification; note (original language) = 甲氧基修饰
  modified_base 16: mod_base = OTHER; note = Methoxy modification; note (original language) = 甲氧基修饰
  modified_base 17: mod_base = OTHER; note = Methoxy modification; note (original language) = 甲氧基修饰
  modified_base 18: mod_base = OTHER; note = Methoxy modification; note (original language) = 甲氧基修饰
  modified_base 19: mod_base = OTHER; note = Methoxy modification; note (original language) = 甲氧基修饰
  misc_feature 1..19: note = synthetic sequence; note (original language) = 合成序列
gtgtgcacttcgcttcaca

SEQ ID NO: 14 - RNA, 21 nt, synthetic construct
  source 1..21: mol_type = other RNA
  modified_base 1: mod_base = OTHER; note = Methoxy modification; note (original language) = 甲氧基修饰
  modified_base 1..2: mod_base = OTHER; note = Thiophosphate ester subunit connection; note (original language) = 硫代磷酸酯亚基连接
  modified_base 2: mod_base = OTHER; note = Fluorinated modification; note (original language) = 氟代修饰
  modified_base 2..3: mod_base = OTHER; note = Thiophosphate ester subunit connection; note (original language) = 硫代磷酸酯亚基连接
  modified_base 3: mod_base = OTHER; note = Methoxy modification; note (original language) = 甲氧基修饰
  modified_base 4: mod_base = OTHER; note = Methoxy modification; note (original language) = 甲氧基修饰
  modified_base 5: mod_base = OTHER; note = Methoxy modification; note (original language) = 甲氧基修饰
  modified_base 6: mod_base = OTHER; note = Agn(Adenosine glycerol nucleic acid); note (original language) = 腺苷甘油核酸
  modified_base 7: mod_base = OTHER; note = Methoxy modification; note (original language) = 甲氧基修饰
  modified_base 8: mod_base = OTHER; note = Fluorinated modification; note (original language) = 氟代修饰
  modified_base 9: mod_base = OTHER; note = Fluorinated modification; note (original language) = 氟代修饰
  modified_base 10: mod_base = OTHER; note = Methoxy modification; note (original language) = 甲氧基修饰
  modified_base 11: mod_base = OTHER; note = Methoxy modification; note (original language) = 甲氧基修饰
  modified_base 12: mod_base = OTHER; note = Methoxy modification; note (original language) = 甲氧基修饰
  modified_base 13: mod_base = OTHER; note = Methoxy modification; note (original language) = 甲氧基修饰
  modified_base 14: mod_base = OTHER; note = Fluorinated modification; note (original language) = 氟代修饰
  modified_base 15: mod_base = OTHER; note = Methoxy modification; note (original language) = 甲氧基修饰
  modified_base 16: mod_base = OTHER; note = Fluorinated modification; note (original language) = 氟代修饰
  modified_base 17: mod_base = OTHER; note = Methoxy modification; note (original language) = 甲氧基修饰
  modified_base 18: mod_base = OTHER; note = Methoxy modification; note (original language) = 甲氧基修饰
  modified_base 19: mod_base = OTHER; note = Methoxy modification; note (original language) = 甲氧基修饰
  modified_base 19..20: mod_base = OTHER; note = Thiophosphate ester subunit connection; note (original language) = 硫代磷酸酯亚基连接
  modified_base 20: mod_base = OTHER; note = Methoxy modification; note (original language) = 甲氧基修饰
  modified_base 20..21: mod_base = OTHER; note = Thiophosphate ester subunit connection; note (original language) = 硫代磷酸酯亚基连接
  modified_base 21: mod_base = OTHER; note = Methoxy modification; note (original language) = 甲氧基修饰
  misc_feature 1..21: note = synthetic sequence; note (original language) = 合成序列
tgtgaagcgaagtgcacactt

SEQ ID NO: 15 - RNA, 23 nt, synthetic construct
  source 1..23: mol_type = other RNA
  modified_base 1: mod_base = OTHER; note = invAb; note (original language) = 反向脱碱基脱氧核糖核苷酸
  modified_base 1..2: mod_base = OTHER; note = Thiophosphate ester subunit connection; note (original language) = 硫代磷酸酯亚基连接
  modified_base 2: mod_base = OTHER; note = Methoxy modification; note (original language) = 甲氧基修饰
  modified_base 3: mod_base = OTHER; note = Methoxy modification; note (original language) = 甲氧基修饰
  modified_base 4: mod_base = OTHER; note = Methoxy modification; note (original language) = 甲氧基修饰
  modified_base 5: mod_base = OTHER; note = Methoxy modification; note (original language) = 甲氧基修饰
  modified_base 6: mod_base = OTHER; note = Methoxy modification; note (original language) = 甲氧基修饰
  modified_base 7: mod_base = OTHER; note = Methoxy modification; note (original language) = 甲氧基修饰
  modified_base 8: mod_base = OTHER; note = Methoxy modification; note (original language) = 甲氧基修饰
  modified_base 9: mod_base = OTHER; note = Methoxy modification; note (original language) = 甲氧基修饰
  modified_base 10: mod_base = OTHER; note = Fluorinated modification; note (original language) = 氟代修饰
  modified_base 11: mod_base = OTHER; note = Fluorinated modification; note (original language) = 氟代修饰
  modified_base 12: mod_base = OTHER; note = Fluorinated modification; note (original language) = 氟代修饰
  modified_base 13: mod_base = OTHER; note = Methoxy modification; note (original language) = 甲氧基修饰
  modified_base 14: mod_base = OTHER; note = Methoxy modification; note (original language) = 甲氧基修饰
  modified_base 15: mod_base = OTHER; note = Methoxy modification; note (original language) = 甲氧基修饰
  modified_base 16: mod_base = OTHER; note = Methoxy modification; note (original language) = 甲氧基修饰
  modified_base 17: mod_base = OTHER; note = Methoxy modification; note (original language) = 甲氧基修饰
  modified_base 18: mod_base = OTHER; note = Methoxy modification; note (original language) = 甲氧基修饰
  modified_base 19: mod_base = OTHER; note = Methoxy modification; note (original language) = 甲氧基修饰
  modified_base 20: mod_base = OTHER; note = Methoxy modification; note (original language) = 甲氧基修饰
  modified_base 21: mod_base = OTHER; note = Methoxy modification; note (original language) = 甲氧基修饰
  modified_base 22: mod_base = OTHER; note = Methoxy modification; note (original language) = 甲氧基修饰
  modified_base 22..23: mod_base = OTHER; note = Thiophosphate ester subunit connection; note (original language) = 硫代磷酸酯亚基连接
  modified_base 23: mod_base = OTHER; note = invAb; note (original language) = 反向脱碱基脱氧核糖核苷酸
  misc_feature 1..23: note = synthetic sequence; note (original language) = 合成序列
ngtggacttctctcaattttctn

SEQ ID NO: 16 - RNA, 21 nt, synthetic construct
  source 1..21: mol_type = other RNA
  modified_base 1: mod_base = OTHER; note = Methoxy modification; note (original language) = 甲氧基修饰
  modified_base 1..2: mod_base = OTHER; note = Thiophosphate ester subunit connection; note (original language) = 硫代磷酸酯亚基连接
  modified_base 2: mod_base = OTHER; note = Fluorinated modification; note (original language) = 氟代修饰
  modified_base 2..3: mod_base = OTHER; note = Thiophosphate ester subunit connection; note (original language) = 硫代磷酸酯亚基连接
  modified_base 3: mod_base = OTHER; note = Methoxy modification; note (original language) = 甲氧基修饰
  modified_base 3..4: mod_base = OTHER; note = Thiophosphate ester subunit connection; note (original language) = 硫代磷酸酯亚基连接
  modified_base 4: mod_base = OTHER; note = Fluorinated modification; note (original language) = 氟代修饰
  modified_base 5: mod_base = OTHER; note = Methoxy modification; note (original language) = 甲氧基修饰
  modified_base 6: mod_base = OTHER; note = Fluorinated modification; note (original language) = 氟代修饰
  modified_base 7: mod_base = OTHER; note = Methoxy modification; note (original language) = 甲氧基修饰
  modified_base 8: mod_base = OTHER; note = Fluorinated modification; note (original language) = 氟代修饰
  modified_base 9: mod_base = OTHER; note = Methoxy modification; note (original language) = 甲氧基修饰
  modified_base 10: mod_base = OTHER; note = Fluorinated modification; note (original language) = 氟代修饰
  modified_base 11: mod_base = OTHER; note = Methoxy modification; note (original language) = 甲氧基修饰
  modified_base 12: mod_base = OTHER; note = Fluorinated modification; note (original language) = 氟代修饰
  modified_base 13: mod_base = OTHER; note = Methoxy modification; note (original language) = 甲氧基修饰
  modified_base 14: mod_base = OTHER; note = Fluorinated modification; note (original language) = 氟代修饰
  modified_base 15: mod_base = OTHER; note = Methoxy modification; note (original language) = 甲氧基修饰
  modified_base 16: mod_base = OTHER; note = Fluorinated modification; note (original language) = 氟代修饰
  modified_base 17: mod_base = OTHER; note = Methoxy modification; note (original language) = 甲氧基修饰
  modified_base 18: mod_base = OTHER; note = Fluorinated modification; note (original language) = 氟代修饰
  modified_base 19: mod_base = OTHER; note = Methoxy modification; note (original language) = 甲氧基修饰
  modified_base 20: mod_base = OTHER; note = Methoxy modification; note (original language) = 甲氧基修饰
  modified_base 20..21: mod_base = OTHER; note = Thiophosphate ester subunit connection; note (original language) = 硫代磷酸酯亚基连接
  modified_base 21: mod_base = OTHER; note = Methoxy modification; note (original language) = 甲氧基修饰
  misc_feature 1..21: note = synthetic sequence; note (original language) = 合成序列
agaaaattgagagaagtccac

SEQ ID NO: 17 - RNA, 23 nt, synthetic construct
  source 1..23: mol_type = other RNA
  modified_base 1: mod_base = OTHER; note = invAb; note (original language) = 反向脱碱基脱氧核糖核苷酸
  modified_base 1..2: mod_base = OTHER; note = Thiophosphate ester subunit connection; note (original language) = 硫代磷酸酯亚基连接
  modified_base 2: mod_base = OTHER; note = Methoxy modification; note (original language) = 甲氧基修饰
  modified_base 3: mod_base = OTHER; note = Methoxy modification; note (original language) = 甲氧基修饰
  modified_base 4: mod_base = OTHER; note = Methoxy modification; note (original language) = 甲氧基修饰
  modified_base 5: mod_base = OTHER; note = Methoxy modification; note (original language) = 甲氧基修饰
  modified_base 6: mod_base = OTHER; note = Methoxy modification; note (original language) = 甲氧基修饰
  modified_base 7: mod_base = OTHER; note = Methoxy modification; note (original language) = 甲氧基修饰
  modified_base 8: mod_base = OTHER; note = Methoxy modification; note (original language) = 甲氧基修饰
  modified_base 9: mod_base = OTHER; note = Methoxy modification; note (original language) = 甲氧基修饰
  modified_base 10: mod_base = OTHER; note = Fluorinated modification; note (original language) = 氟代修饰
  modified_base 11: mod_base = OTHER; note = Fluorinated modification; note (original language) = 氟代修饰
  modified_base 12: mod_base = OTHER; note = Fluorinated modification; note (original language) = 氟代修饰
  modified_base 13: mod_base = OTHER; note = Methoxy modification; note (original language) = 甲氧基修饰
  modified_base 14: mod_base = OTHER; note = Methoxy modification; note (original language) = 甲氧基修饰
  modified_base 15: mod_base = OTHER; note = Methoxy modification; note (original language) = 甲氧基修饰
  modified_base 16: mod_base = OTHER; note = Methoxy modification; note (original language) = 甲氧基修饰
  modified_base 17: mod_base = OTHER; note = Methoxy modification; note (original language) = 甲氧基修饰
  modified_base 18: mod_base = OTHER; note = Methoxy modification; note (original language) = 甲氧基修饰
  modified_base 19: mod_base = OTHER; note = Methoxy modification; note (original language) = 甲氧基修饰
  modified_base 20: mod_base = OTHER; note = Methoxy modification; note (original language) = 甲氧基修饰
  modified_base 21: mod_base = OTHER; note = Methoxy modification; note (original language) = 甲氧基修饰
  modified_base 22: mod_base = OTHER; note = Methoxy modification; note (original language) = 甲氧基修饰
  modified_base 22..23: mod_base = OTHER; note = Thiophosphate ester subunit connection; note (original language) = 硫代磷酸酯亚基连接
  modified_base 23: mod_base = OTHER; note = invAb; note (original language) = 反向脱碱基脱氧核糖核苷酸
  misc_feature 1..23: note = synthetic sequence; note (original language) = 合成序列
ncgctgtaggcataaattggtan

SEQ ID NO: 18 - RNA, 21 nt, synthetic construct
  source 1..21: mol_type = other RNA
  modified_base 1: mod_base = OTHER; note = Methoxy modification; note (original language) = 甲氧基修饰
  modified_base 1..2: mod_base = OTHER; note = Thiophosphate ester subunit connection; note (original language) = 硫代磷酸酯亚基连接
  modified_base 2: mod_base = OTHER; note = Fluorinated modification; note (original language) = 氟代修饰
  modified_base 2..3: mod_base = OTHER; note = Thiophosphate ester subunit connection; note (original language) = 硫代磷酸酯亚基连接
  modified_base 3: mod_base = OTHER; note = Methoxy modification; note (original language) = 甲氧基修饰
  modified_base 3..4: mod_base = OTHER; note = Thiophosphate ester subunit connection; note (original language) = 硫代磷酸酯亚基连接
  modified_base 4: mod_base = OTHER; note = Fluorinated modification; note (original language) = 氟代修饰
  modified_base 5: mod_base = OTHER; note = Methoxy modification; note (original language) = 甲氧基修饰
  modified_base 6: mod_base = OTHER; note = Fluorinated modification; note (original language) = 氟代修饰
  modified_base 7: mod_base = OTHER; note = Methoxy modification; note (original language) = 甲氧基修饰
  modified_base 8: mod_base = OTHER; note = Fluorinated modification; note (original language) = 氟代修饰
  modified_base 9: mod_base = OTHER; note = Methoxy modification; note (original language) = 甲氧基修饰
  modified_base 10: mod_base = OTHER; note = Fluorinated modification; note (original language) = 氟代修饰
  modified_base 11: mod_base = OTHER; note = Methoxy modification; note (original language) = 甲氧基修饰
  modified_base 12: mod_base = OTHER; note = Fluorinated modification; note (original language) = 氟代修饰
  modified_base 13: mod_base = OTHER; note = Methoxy modification; note (original language) = 甲氧基修饰
  modified_base 14: mod_base = OTHER; note = Fluorinated modification; note (original language) = 氟代修饰
  modified_base 15: mod_base = OTHER; note = Methoxy modification; note (original language) = 甲氧基修饰
  modified_base 16: mod_base = OTHER; note = Fluorinated modification; note (original language) = 氟代修饰
  modified_base 17: mod_base = OTHER; note = Methoxy modification; note (original language) = 甲氧基修饰
  modified_base 18: mod_base = OTHER; note = Fluorinated modification; note (original language) = 氟代修饰
  modified_base 19: mod_base = OTHER; note = Methoxy modification; note (original language) = 甲氧基修饰
  modified_base 20: mod_base = OTHER; note = Methoxy modification; note (original language) = 甲氧基修饰
  modified_base 20..21: mod_base = OTHER; note = Thiophosphate ester subunit connection; note (original language) = 硫代磷酸酯亚基连接
  modified_base 21: mod_base = OTHER; note = Methoxy modification; note (original language) = 甲氧基修饰
  misc_feature 1..21: note = synthetic sequence; note (original language) = 合成序列
taccaatttatgcctacagcg

SEQ ID NO: 19 - RNA, 17 nt, synthetic construct
  source 1..17: mol_type = other RNA
  modified_base 1: mod_base = OTHER; note = Methoxy modification; note (original language) = 甲氧基修饰
  modified_base 1..2: mod_base = OTHER; note = Thiophosphate ester subunit connection; note (original language) = 硫代磷酸酯亚基连接
  modified_base 2: mod_base = OTHER; note = Methoxy modification; note (original language) = 甲氧基修饰
  modified_base 2..3: mod_base = OTHER; note = Thiophosphate ester subunit connection; note (original language) = 硫代磷酸酯亚基连接
  modified_base 3: mod_base = OTHER; note = Methoxy modification; note (original language) = 甲氧基修饰
  modified_base 4: mod_base = OTHER; note = Methoxy modification; note (original language) = 甲氧基修饰
  modified_base 5: mod_base = OTHER; note = Fluorinated modification; note (original language) = 氟代修饰
  modified_base 6: mod_base = OTHER; note = Fluorinated modification; note (original language) = 氟代修饰
  modified_base 7: mod_base = OTHER; note = Fluorinated modification; note (original language) = 氟代修饰
  modified_base 8: mod_base = OTHER; note = Methoxy modification; note (original language) = 甲氧基修饰
  modified_base 9: mod_base = OTHER; note = Methoxy modification; note (original language) = 甲氧基修饰
  modified_base 10: mod_base = OTHER; note = Methoxy modification; note (original language) = 甲氧基修饰
  modified_base 11: mod_base = OTHER; note = Methoxy modification; note (original language) = 甲氧基修饰
  modified_base 12: mod_base = OTHER; note = Methoxy modification; note (original language) = 甲氧基修饰
  modified_base 13: mod_base = OTHER; note = Methoxy modification; note (original language) = 甲氧基修饰
  modified_base 14: mod_base = OTHER; note = Methoxy modification; note (original language) = 甲氧基修饰
  modified_base 15: mod_base = OTHER; note = Methoxy modification; note (original language) = 甲氧基修饰
  modified_base 16: mod_base = OTHER; note = Methoxy modification; note (original language) = 甲氧基修饰
  modified_base 17: mod_base = OTHER; note = Methoxy modification; note (original language) = 甲氧基修饰
  misc_feature 1..17: note = synthetic sequence; note (original language) = 合成序列
gtgcacttcgcttcaca

SEQ ID NO: 20 - RNA, 22 nt, synthetic construct
  source 1..22: mol_type = other RNA
  modified_base 1: mod_base = OTHER; note = Methoxy modification; note (original language) = 甲氧基修饰
  modified_base 1..2: mod_base = OTHER; note = Thiophosphate ester subunit connection; note (original language) = 硫代磷酸酯亚基连接
  modified_base 2: mod_base = OTHER; note = Fluorinated modification; note (original language) = 氟代修饰
  modified_base 2..3: mod_base = OTHER; note = Thiophosphate ester subunit connection; note (original language) = 硫代磷酸酯亚基连接
  modified_base 3: mod_base = OTHER; note = Methoxy modification; note (original language) = 甲氧基修饰
  modified_base 4: mod_base = OTHER; note = Methoxy modification; note (original language) = 甲氧基修饰
  modified_base 5: mod_base = OTHER; note = Methoxy modification; note (original language) = 甲氧基修饰
  modified_base 6: mod_base = OTHER; note = Methoxy modification; note (original language) = 甲氧基修饰
  modified_base 7: mod_base = OTHER; note = Methoxy modification; note (original language) = 甲氧基修饰
  modified_base 8: mod_base = OTHER; note = Methoxy modification; note (original language) = 甲氧基修饰
  modified_base 9: mod_base = OTHER; note = Methoxy modification; note (original language) = 甲氧基修饰
  modified_base 10: mod_base = OTHER; note = Methoxy modification; note (original language) = 甲氧基修饰
  modified_base 11: mod_base = OTHER; note = Methoxy modification; note (original language) = 甲氧基修饰
  modified_base 12: mod_base = OTHER; note = Methoxy modification; note (original language) = 甲氧基修饰
  modified_base 13: mod_base = OTHER; note = Methoxy modification; note (original language) = 甲氧基修饰
  modified_base 14: mod_base = OTHER; note = Fluorinated modification; note (original language) = 氟代修饰
  modified_base 15: mod_base = OTHER; note = Methoxy modification; note (original language) = 甲氧基修饰
  modified_base 16: mod_base = OTHER; note = Fluorinated modification; note (original language) = 氟代修饰
  modified_base 17: mod_base = OTHER; note = Methoxy modification; note (original language) = 甲氧基修饰
  modified_base 18: mod_base = OTHER; note = Methoxy modification; note (original language) = 甲氧基修饰
  modified_base 19: mod_base = OTHER; note = Methoxy modification; note (original language) = 甲氧基修饰
  modified_base 19..20: mod_base = OTHER; note = Thiophosphate ester subunit connection; note (original language) = 硫代磷酸酯亚基连接
  modified_base 20: mod_base = OTHER; note = Methoxy modification; note (original language) = 甲氧基修饰
  modified_base 20..21: mod_base = OTHER; note = Thiophosphate ester subunit connection; note (original language) = 硫代磷酸酯亚基连接
  modified_base 21: mod_base = OTHER; note = Methoxy modification; note (original language) = 甲氧基修饰
  modified_base 22: mod_base = OTHER; note = Fluorinated modification; note (original language) = 氟代修饰
  misc_feature 1..22: note = synthetic sequence; note (original language) = 合成序列
tgtgaagcgaagtgcacacggt

SEQ ID NO: 21 - RNA, 17 nt, synthetic construct
  source 1..17: mol_type = other RNA
  modified_base 1: mod_base = OTHER; note = Methoxy modification; note (original language) = 甲氧基修饰
  modified_base 1..2: mod_base = OTHER; note = Thiophosphate ester subunit connection; note (original language) = 硫代磷酸酯亚基连接
  modified_base 2: mod_base = OTHER; note = Methoxy modification; note (original language) = 甲氧基修饰
  modified_base 2..3: mod_base = OTHER; note = Thiophosphate ester subunit connection; note (original language) = 硫代磷酸酯亚基连接
  modified_base 3: mod_base = OTHER; note = Methoxy modification; note (original language) = 甲氧基修饰
  modified_base 4: mod_base = OTHER; note = Methoxy modification; note (original language) = 甲氧基修饰
  modified_base 5: mod_base = OTHER; note = Fluorinated modification; note (original language) = 氟代修饰
  modified_base 6: mod_base = OTHER; note = Fluorinated modification; note (original language) = 氟代修饰
  modified_base 7: mod_base = OTHER; note = Fluorinated modification; note (original language) = 氟代修饰
  modified_base 8: mod_base = OTHER; note = Methoxy modification; note (original language) = 甲氧基修饰
  modified_base 9: mod_base = OTHER; note = Methoxy modification; note (original language) = 甲氧基修饰
  modified_base 10: mod_base = OTHER; note = Methoxy modification; note (original language) = 甲氧基修饰
  modified_base 11: mod_base = OTHER; note = Methoxy modification; note (original language) = 甲氧基修饰
  modified_base 12: mod_base = OTHER; note = Methoxy modification; note (original language) = 甲氧基修饰
  modified_base 13: mod_base = OTHER; note = Methoxy modification; note (original language) = 甲氧基修饰
  modified_base 14: mod_base = OTHER; note = Methoxy modification; note (original language) = 甲氧基修饰
  modified_base 15: mod_base = OTHER; note = Methoxy modification; note (original language) = 甲氧基修饰
  modified_base 16: mod_base = OTHER; note = Methoxy modification; note (original language) = 甲氧基修饰
  modified_base 17: mod_base = OTHER; note = Methoxy modification; note (original language) = 甲氧基修饰
  misc_feature 1..17: note = synthetic sequence; note (original language) = 合成序列
gtgcacttcgcttcaca

SEQ ID NO: 22 - RNA, 22 nt, synthetic construct
  source 1..22: mol_type = other RNA
  modified_base 1: mod_base = OTHER; note = Methoxy modification; note (original language) = 甲氧基修饰
  modified_base 1..2: mod_base = OTHER; note = Thiophosphate ester subunit connection; note (original language) = 硫代磷酸酯亚基连接
  modified_base 2: mod_base = OTHER; note = Fluorinated modification; note (original language) = 氟代修饰
  modified_base 2..3: mod_base = OTHER; note = Thiophosphate ester subunit connection; note (original language) = 硫代磷酸酯亚基连接
  modified_base 3: mod_base = OTHER; note = Methoxy modification; note (original language) = 甲氧基修饰
  modified_base 4: mod_base = OTHER; note = Methoxy modification; note (original language) = 甲氧基修饰
  modified_base 5: mod_base = OTHER; note = Agn(Adenosine glycerol nucleic acid); note (original language) = 腺苷甘油核酸
  modified_base 6: mod_base = OTHER; note = Methoxy modification; note (original language) = 甲氧基修饰
  modified_base 7: mod_base = OTHER; note = Methoxy modification; note (original language) = 甲氧基修饰
  modified_base 8: mod_base = OTHER; note = Methoxy modification; note (original language) = 甲氧基修饰
  modified_base 9: mod_base = OTHER; note = Methoxy modification; note (original language) = 甲氧基修饰
  modified_base 10: mod_base = OTHER; note = Methoxy modification; note (original language) = 甲氧基修饰
  modified_base 11: mod_base = OTHER; note = Methoxy modification; note (original language) = 甲氧基修饰
  modified_base 12: mod_base = OTHER; note = Methoxy modification; note (original language) = 甲氧基修饰
  modified_base 13: mod_base = OTHER; note = Methoxy modification; note (original language) = 甲氧基修饰
  modified_base 14: mod_base = OTHER; note = Fluorinated modification; note (original language) = 氟代修饰
  modified_base 15: mod_base = OTHER; note = Methoxy modification; note (original language) = 甲氧基修饰
  modified_base 16: mod_base = OTHER; note = Fluorinated modification; note (original language) = 氟代修饰
  modified_base 17: mod_base = OTHER; note = Methoxy modification; note (original language) = 甲氧基修饰
  modified_base 18: mod_base = OTHER; note = Methoxy modification; note (original language) = 甲氧基修饰
  modified_base 19: mod_base = OTHER; note = Methoxy modification; note (original language) = 甲氧基修饰
  modified_base 19..20: mod_base = OTHER; note = Thiophosphate ester subunit connection; note (original language) = 硫代磷酸酯亚基连接
  modified_base 20: mod_base = OTHER; note = Methoxy modification; note (original language) = 甲氧基修饰
  modified_base 20..21: mod_base = OTHER; note = Thiophosphate ester subunit connection; note (original language) = 硫代磷酸酯亚基连接
  modified_base 21: mod_base = OTHER; note = Methoxy modification; note (original language) = 甲氧基修饰
  modified_base 22: mod_base = OTHER; note = Fluorinated modification; note (original language) = 氟代修饰
  misc_feature 1..22: note = synthetic sequence; note (original language) = 合成序列
tgtgaagcgaagtgcacacggt

SEQ ID NO: 23 - RNA, 17 nt, synthetic construct
  source 1..17: mol_type = other RNA
  modified_base 1: mod_base = OTHER; note = Methoxy modification; note (original language) = 甲氧基修饰
  modified_base 1..2: mod_base = OTHER; note = Thiophosphate ester subunit connection; note (original language) = 硫代磷酸酯亚基连接
  modified_base 2: mod_base = OTHER; note = Methoxy modification; note (original language) = 甲氧基修饰
  modified_base 2..3: mod_base = OTHER; note = Thiophosphate ester subunit connection; note (original language) = 硫代磷酸酯亚基连接
  modified_base 3: mod_base = OTHER; note = Methoxy modification; note (original language) = 甲氧基修饰
  modified_base 4: mod_base = OTHER; note = Methoxy modification; note (original language) = 甲氧基修饰
  modified_base 5: mod_base = OTHER; note = Fluorinated modification; note (original language) = 氟代修饰
  modified_base 6: mod_base = OTHER; note = Fluorinated modification; note (original language) = 氟代修饰
  modified_base 7: mod_base = OTHER; note = Fluorinated modification; note (original language) = 氟代修饰
  modified_base 8: mod_base = OTHER; note = Methoxy modification; note (original language) = 甲氧基修饰
  modified_base 9: mod_base = OTHER; note = Methoxy modification; note (original language) = 甲氧基修饰
  modified_base 10: mod_base = OTHER; note = Methoxy modification; note (original language) = 甲氧基修饰
  modified_base 11: mod_base = OTHER; note = Methoxy modification; note (original language) = 甲氧基修饰
  modified_base 12: mod_base = OTHER; note = Methoxy modification; note (original language) = 甲氧基修饰
  modified_base 13: mod_base = OTHER; note = Methoxy modification; note (original language) = 甲氧基修饰
  modified_base 14: mod_base = OTHER; note = Methoxy modification; note (original language) = 甲氧基修饰
  modified_base 15: mod_base = OTHER; note = Methoxy modification; note (original language) = 甲氧基修饰
  modified_base 16: mod_base = OTHER; note = Methoxy modification; note (original language) = 甲氧基修饰
  modified_base 17: mod_base = OTHER; note = Methoxy modification; note (original language) = 甲氧基修饰
  misc_feature 1..17: note = synthetic sequence; note (original language) = 合成序列
gtgcacttcgcttcaca

SEQ ID NO: 24 - RNA, 22 nt, synthetic construct
  source 1..22: mol_type = other RNA
  modified_base 1: mod_base = OTHER; note = Methoxy modification; note (original language) = 甲氧基修饰
  modified_base 1..2: mod_base = OTHER; note = Thiophosphate ester subunit connection; note (original language) = 硫代磷酸酯亚基连接
  modified_base 2: mod_base = OTHER; note = Fluorinated modification; note (original language) = 氟代修饰
  modified_base 2..3: mod_base = OTHER; note = Thiophosphate ester subunit connection; note (original language) = 硫代磷酸酯亚基连接
  modified_base 3: mod_base = OTHER; note = Methoxy modification; note (original language) = 甲氧基修饰
  modified_base 4: mod_base = OTHER; note = Methoxy modification; note (original language) = 甲氧基修饰
  modified_base 5: mod_base = OTHER; note = Methoxy modification; note (original language) = 甲氧基修饰
  modified_base 6: mod_base = OTHER; note = Agn(Adenosine glycerol nucleic acid); note (original language) = 腺苷甘油核酸
  modified_base 7: mod_base = OTHER; note = Methoxy modification; note (original language) = 甲氧基修饰
  modified_base 8: mod_base = OTHER; note = Methoxy modification; note (original language) = 甲氧基修饰
  modified_base 9: mod_base = OTHER; note = Methoxy modification; note (original language) = 甲氧基修饰
  modified_base 10: mod_base = OTHER; note = Methoxy modification; note (original language) = 甲氧基修饰
  modified_base 11: mod_base = OTHER; note = Methoxy modification; note (original language) = 甲氧基修饰
  modified_base 12: mod_base = OTHER; note = Methoxy modification; note (original language) = 甲氧基修饰
  modified_base 13: mod_base = OTHER; note = Methoxy modification; note (original language) = 甲氧基修饰
  modified_base 14: mod_base = OTHER; note = Fluorinated modification; note (original language) = 氟代修饰
  modified_base 15: mod_base = OTHER; note = Methoxy modification; note (original language) = 甲氧基修饰
  modified_base 16: mod_base = OTHER; note = Fluorinated modification; note (original language) = 氟代修饰
  modified_base 17: mod_base = OTHER; note = Methoxy modification; note (original language) = 甲氧基修饰
  modified_base 18: mod_base = OTHER; note = Methoxy modification; note (original language) = 甲氧基修饰
  modified_base 19: mod_base = OTHER; note = Methoxy modification; note (original language) = 甲氧基修饰
  modified_base 19..20: mod_base = OTHER; note = Thiophosphate ester subunit connection; note (original language) = 硫代磷酸酯亚基连接
  modified_base 20: mod_base = OTHER; note = Methoxy modification; note (original language) = 甲氧基修饰
  modified_base 20..21: mod_base = OTHER; note = Thiophosphate ester subunit connection; note (original language) = 硫代磷酸酯亚基连接
  modified_base 21: mod_base = OTHER; note = Methoxy modification; note (original language) = 甲氧基修饰
  modified_base 22: mod_base = OTHER; note = Fluorinated modification; note (original language) = 氟代修饰
  misc_feature 1..22: note = synthetic sequence; note (original language) = 合成序列
tgtgaagcgaagtgcacacggt

SEQ ID NO: 25 - DNA, 24 bp, synthetic construct
  source 1..24: mol_type = other DNA
  misc_feature 1..24: note = synthetic sequence; note (original language) = 合成序列
tcgtcgttttgtcgttttgtcgtt

SEQ ID NO: 26 - DNA, 22 bp, synthetic construct
  source 1..22: mol_type = other DNA
  misc_feature 1..22: note = synthetic sequence; note (original language) = 合成序列
tgactgtgaacgttcgagatga